European Patent Application EP 4 379 726 A1, published June 5, 2024. Title: The method for predicting the occurrence of the off-target toxicity caused by similarity between a target epitope and putative off-target epitopes. Applicant: Ardigen S.A. Application EP 22461636.7, filed December 2, 2022. The sequence listing filed with the application follows.

SEQUENCE LISTING (250 sequences)

SEQ ID NO: 1 - protein, 9 aa, Homo sapiens
EVDPIGHLY

SEQ ID NO: 2 - protein, 9 aa, Homo sapiens
ESDPIVAQY

SEQ ID NO: 3 - protein, 9 aa, Homo sapiens
EVDPIGHLY

SEQ ID NO: 4 - protein, 9 aa, Homo sapiens
EVDPIGHVY

SEQ ID NO: 5 - protein, 9 aa, Homo sapiens
EVDPIRHYY

SEQ ID NO: 6 - protein, 9 aa, Homo sapiens
EMDPVTQLY

SEQ ID NO: 7 - protein, 9 aa, Homo sapiens
KSDPICVLY

SEQ ID NO: 8 - protein, 9 aa, Homo sapiens
EVGPIFHLY

SEQ ID NO: 9 - protein, 9 aa, Homo sapiens
EEHPILFLY

SEQ ID NO: 10 - protein, 9 aa, Homo sapiens
AVDPIKDMY

SEQ ID NO: 11 - protein, 9 aa, Homo sapiens
EVEPFKSLY

SEQ ID NO: 12 - protein, 9 aa, Homo sapiens
SSDPIWDLY

SEQ ID NO: 13 - protein, 9 aa, Homo sapiens
KMVELVHFL

SEQ ID NO: 14 - protein, 9 aa, Homo sapiens
KVAELVHFL

SEQ ID NO: 15 - protein, 9 aa, Homo sapiens
KVDELAHFL

SEQ ID NO: 16 - protein, 9 aa, Homo sapiens
KVADLIHFL

SEQ ID NO: 17 - protein, 9 aa, Homo sapiens
KVAKLVHFL

SEQ ID NO: 18 - protein, 9 aa, Homo sapiens
KVAELVRFL

SEQ ID NO: 19 - protein, 9 aa, Homo sapiens
KVAELVHFL

SEQ ID NO: 20 - protein, 9 aa, Homo sapiens
KVTDLVQFL

SEQ ID NO: 21 - protein, 9 aa, Homo sapiens
KIIDLVHLL

SEQ ID NO: 22 - protein, 9 aa, Homo sapiens
KMAELVHFL

SEQ ID NO: 23 - protein, 9 aa, Homo sapiens
KSGSLVQFL

SEQ ID NO: 24 - protein, 9 aa, Homo sapiens
KTNMLVQFL

SEQ ID NO: 25 - protein, 9 aa, Homo sapiens
KTKMLVQFL

SEQ ID NO: 26 - protein, 9 aa, Homo sapiens
KVGLLEQFL

SEQ ID NO: 27 - protein, 9 aa, Homo sapiens
KVIILVHYL

SEQ ID NO: 28 - protein, 9 aa, Homo sapiens
KVAFLVNFM

SEQ ID NO: 29 - protein, 9 aa, Homo sapiens
KTGELVQFL

SEQ ID NO: 30 - protein, 9 aa, Homo sapiens
KVLEFVAKL

SEQ ID NO: 31 - protein, 9 aa, Homo sapiens
KVVSLVHFL

SEQ ID NO: 32 - protein, 9 aa, Homo sapiens
KVDELARFL

SEQ ID NO: 33 - protein, 9 aa, Homo sapiens
KMALEIVFL

SEQ ID NO: 34 - protein, 9 aa, Homo sapiens
QAAELEREL

SEQ ID NO: 35 - protein, 9 aa, Homo sapiens
AVAVLGGFF

SEQ ID NO: 36 - protein, 9 aa, Homo sapiens
RVTALVHRQ

SEQ ID NO: 37 - protein, 9 aa, Homo sapiens
KKIEGVHFT

SEQ ID NO: 38 - protein, 9 aa, Homo sapiens
KVVELLSEE

SEQ ID NO: 39 - protein, 9 aa, Homo sapiens
YRAELVGEL

SEQ ID NO: 40 - protein, 9 aa, Homo sapiens
KGAEAVEFF

SEQ ID NO: 41 - protein, 9 aa, Homo sapiens
MVANLVPFT

SEQ ID NO: 42 - protein, 9 aa, Homo sapiens
KFYEEVHDL

SEQ ID NO: 43 - protein, 9 aa, Homo sapiens
VVAERVLYL

SEQ ID NO: 44 - protein, 9 aa, Homo sapiens
KVAPLVFFH

SEQ ID NO: 45 - protein, 9 aa, Homo sapiens
EVAELYEQL

SEQ ID NO: 46 - protein, 9 aa, Homo sapiens
KVLALEHLL

SEQ ID NO: 47 - protein, 9 aa, Homo sapiens
QVAERVEAL

SEQ ID NO: 48 - protein, 9 aa, Homo sapiens
EVAWLVYVL

SEQ ID NO: 49 - protein, 9 aa, Homo sapiens
CVAELIQQL

SEQ ID NO: 50 - protein, 9 aa, Homo sapiens
CMEELVELL

SEQ ID NO: 51 - protein, 9 aa, Homo sapiens
VVAVLFIFL

SEQ ID NO: 52 - protein, 9 aa, Homo sapiens
KEELLVHLL

SEQ ID NO: 53 - protein, 9 aa, Homo sapiens
KVAPLEAKL

SEQ ID NO: 54 - protein, 9 aa, Homo sapiens
KVVSLVHFL

SEQ ID NO: 55 - protein, 9 aa, Homo sapiens
SVADLAHVL

SEQ ID NO: 56 - protein, 9 aa, Homo sapiens
KLVELEHTL

SEQ ID NO: 57 - protein, 9 aa, Homo sapiens
MVDELVLLL

SEQ ID NO: 58 - protein, 9 aa, Homo sapiens
KVAELVQFL

SEQ ID NO: 59 - protein, 9 aa, Homo sapiens
KVAELVEFL

SEQ ID NO: 60 - protein, 9 aa, Homo sapiens
KVAELVHFL

SEQ ID NO: 61 - protein, 9 aa, Homo sapiens
KIIDLVHLL

SEQ ID NO: 62 - protein, 9 aa, Homo sapiens
KVAELVHFL

SEQ ID NO: 63 - protein, 9 aa, Homo sapiens
KVAELVRFL

SEQ ID NO: 64 - protein, 9 aa, Homo sapiens
KVDELAHFL

SEQ ID NO: 65 - protein, 9 aa, Homo sapiens
KVTDLVQFL

SEQ ID NO: 66 - protein, 9 aa, Homo sapiens
KVAELVHFL

SEQ ID NO: 67 - protein, 9 aa, Homo sapiens
KMVELVHFL

SEQ ID NO: 68 - protein, 9 aa, Homo sapiens
KMAELVHFL

SEQ ID NO: 69 - protein, 9 aa, Homo sapiens
KMVELVHFL

SEQ ID NO: 70 - protein, 9 aa, Homo sapiens
KLAELARQL

SEQ ID NO: 71 - protein, 9 aa, Homo sapiens
AIAGLVVFL

SEQ ID NO: 72 - protein, 9 aa, Homo sapiens
RVADLVHIL

SEQ ID NO: 73 - protein, 9 aa, Homo sapiens
EDDPKVHLE

SEQ ID NO: 74 - protein, 9 aa, Homo sapiens
TLDPHGHLI

SEQ ID NO: 75 - protein, 9 aa, Homo sapiens
AVSPDGTLY

SEQ ID NO: 76 - protein, 9 aa, Homo sapiens
EYDPEGHLT

SEQ ID NO: 77 - protein, 9 aa, Homo sapiens
GVDPVGRLL

SEQ ID NO: 78 - protein, 9 aa, Homo sapiens
EVLQIEHSY

SEQ ID NO: 79 - protein, 9 aa, Homo sapiens
EEDGIRRLY

SEQ ID NO: 80 - protein, 9 aa, Homo sapiens
EVDELLHIY

SEQ ID NO: 81 - protein, 9 aa, Homo sapiens
EVDPSKHSF

SEQ ID NO: 82 - protein, 9 aa, Homo sapiens
ESDPIVAQY

SEQ ID NO: 83 - protein, 9 aa, Homo sapiens
ESLPKDHLY

SEQ ID NO: 84 - protein, 9 aa, Homo sapiens
VVQEIGHLI

SEQ ID NO: 85 - protein, 9 aa, Homo sapiens
SVLPIAHLN

SEQ ID NO: 86 - protein, 9 aa, Homo sapiens
ENFPIGHLK

SEQ ID NO: 87 - protein, 9 aa, Homo sapiens
HVDPVGPLD

SEQ ID NO: 88 - protein, 9 aa, Homo sapiens
EVDPEGLVI

SEQ ID NO: 89 - protein, 9 aa, Homo sapiens
EVNPAAHLT

SEQ ID NO: 90 - protein, 9 aa, Homo sapiens
KVSMEGHLY

SEQ ID NO: 91 - protein, 9 aa, Homo sapiens
SPDPIGHNP

SEQ ID NO: 92 - protein, 9 aa, Homo sapiens
TVDGIGALP

SEQ ID NO: 93 - protein, 9 aa, Homo sapiens
GRRLLGHLY

SEQ ID NO: 94 - protein, 9 aa, Homo sapiens
ENDPSGFLQ

SEQ ID NO: 95 - protein, 9 aa, Homo sapiens
VVPPIRLLY

SEQ ID NO: 96 - protein, 9 aa, Homo sapiens
IVPPIRPLY

SEQ ID NO: 97 - protein, 9 aa, Homo sapiens
EADGGGHLD

SEQ ID NO: 98 - protein, 9 aa, Homo sapiens
EGDGRGHLD

SEQ ID NO: 99 - protein, 9 aa, Homo sapiens
PLDPEGHLH

SEQ ID NO: 100 - protein, 9 aa, Homo sapiens
GNDPAIHLY

SEQ ID NO: 101 - protein, 9 aa, Homo sapiens
EVDSKAHLR

SEQ ID NO: 102 - protein, 9 aa, Homo sapiens
EVDPDEGLF

SEQ ID NO: 103 - protein, 9 aa, Homo sapiens
EVRPDGLGG

SEQ ID NO: 104 - protein, 9 aa, Homo sapiens
EVRPDGHGG

SEQ ID NO: 105 - protein, 9 aa, Homo sapiens
PVDPISHDL

SEQ ID NO: 106 - protein, 9 aa, Homo sapiens
EGVPSGHLY

SEQ ID NO: 107 - protein, 9 aa, Homo sapiens
EVDLCAHGH

SEQ ID NO: 108 - protein, 9 aa, Homo sapiens
EESTIGHLK

SEQ ID NO: 109 - protein, 9 aa, Homo sapiens
EEDPLVHLS

SEQ ID NO: 110 - protein, 9 aa, Homo sapiens
CMDCYNHLY

SEQ ID NO: 111 - protein, 9 aa, Homo sapiens
EVHLIGMVR

SEQ ID NO: 112 - protein, 9 aa, Homo sapiens
EVDPTSNTY

SEQ ID NO: 113 - protein, 9 aa, Homo sapiens
VLDFITHLY

SEQ ID NO: 114 - protein, 9 aa, Homo sapiens
ELDPTFGLY

SEQ ID NO: 115 - protein, 9 aa, Homo sapiens
KVDGFTHLY

SEQ ID NO: 116 - protein, 9 aa, Homo sapiens
GNDPAIHLY

SEQ ID NO: 117 - protein, 9 aa, Homo sapiens
GNDPAIHLY

SEQ ID NO: 118 - protein, 9 aa, Homo sapiens
VVDPSSNLY

SEQ ID NO: 119 - protein, 9 aa, Homo sapiens
ERDKIFLLY

SEQ ID NO: 120 - protein, 9 aa, Homo sapiens
RVDQNGVLY

SEQ ID NO: 121 - protein, 9 aa, Homo sapiens
EVDEITLWY

SEQ ID NO: 122 - protein, 9 aa, Homo sapiens
ESDPIVAQY

SEQ ID NO: 123 - protein, 9 aa, Homo sapiens
WVDPIDSTY

SEQ ID NO: 124 - protein, 9 aa, Homo sapiens
SVDKIEVLY

SEQ ID NO: 125 - protein, 9 aa, Homo sapiens
KVDGIYLLY

SEQ ID NO: 126 - protein, 9 aa, Homo sapiens
EVDPDTILK

SEQ ID NO: 127 - protein, 9 aa, Homo sapiens
EVGPIFHLY

SEQ ID NO: 128 - protein, 9 aa, Homo sapiens
TVDENGRLY

SEQ ID NO: 129 - protein, 9 aa, Homo sapiens
VVDNLQHLY

SEQ ID NO: 130 - protein, 9 aa, Homo sapiens
EMDPVTQLY

SEQ ID NO: 131 - protein, 9 aa, Homo sapiens
EVDVPIKLY

SEQ ID NO: 132 - protein, 9 aa, Homo sapiens
FVDPGERLY

SEQ ID NO: 133 - protein, 9 aa, Homo sapiens
FINRGEYEI

SEQ ID NO: 134 - protein, 9 aa, Homo sapiens
TMNPLIYNI

SEQ ID NO: 135 - protein, 9 aa, Homo sapiens
FFYKFGLEI

SEQ ID NO: 136 - protein, 9 aa, Homo sapiens
FAPKFIFEA

SEQ ID NO: 137 - protein, 9 aa, Homo sapiens
FVEKFSIEI

SEQ ID NO: 138 - protein, 9 aa, Homo sapiens
FTYKFAEEI

SEQ ID NO: 139 - protein, 9 aa, Homo sapiens
ADNIFIYES

SEQ ID NO: 140 - protein, 9 aa, Homo sapiens
FDAKIIYEK

SEQ ID NO: 141 - protein, 9 aa, Homo sapiens
FMNSFLEEH

SEQ ID NO: 142 - protein, 9 aa, Homo sapiens
ILNKFIPDI

SEQ ID NO: 143 - protein, 9 aa, Homo sapiens
RTNKFIKEL

SEQ ID NO: 144 - protein, 9 aa, Homo sapiens
KTNKFIKEL

SEQ ID NO: 145 - protein, 9 aa, Homo sapiens
RTNKFIKEL

SEQ ID NO: 146 - protein, 9 aa, Homo sapiens
LKNKWIGEI

SEQ ID NO: 147 - protein, 9 aa, Homo sapiens
FMKRFSYES

SEQ ID NO: 148 - protein, 9 aa, Homo sapiens
FANKEPYEN

SEQ ID NO: 149 - protein, 9 aa, Homo sapiens
EINKKIYKI

SEQ ID NO: 150 - protein, 9 aa, Homo sapiens
VANGFIEEI

SEQ ID NO: 151 - protein, 9 aa, Homo sapiens
LMNLFTYEK

SEQ ID NO: 152 - protein, 9 aa, Homo sapiens
RMNGIIYEI

SEQ ID NO: 153 - protein, 9 aa, Homo sapiens
FENKHGHGI

SEQ ID NO: 154 - protein, 9 aa, Homo sapiens
DTNREIYEI

SEQ ID NO: 155 - protein, 9 aa, Homo sapiens
SKNKFIEQI

SEQ ID NO: 156 - protein, 9 aa, Homo sapiens
AKRKSIYEI

SEQ ID NO: 157 - protein, 9 aa, Homo sapiens
MMNPFIYSL

SEQ ID NO: 158 - protein, 9 aa, Homo sapiens
MLNPFIYST

SEQ ID NO: 159 - protein, 9 aa, Homo sapiens
EINKKIYKI

SEQ ID NO: 160 - protein, 9 aa, Homo sapiens
FLVMFIYSI

SEQ ID NO: 161 - protein, 9 aa, Homo sapiens
CANKFIDHI

SEQ ID NO: 162 - protein, 9 aa, Homo sapiens
MMNPFIYRL

SEQ ID NO: 163 - protein, 9 aa, Homo sapiens
MMNPFIYSL

SEQ ID NO: 164 - protein, 9 aa, Homo sapiens
MMNPFIYSL

SEQ ID NO: 165 - protein, 9 aa, Homo sapiens
MMNPFIYSL

SEQ ID NO: 166 - protein, 9 aa, Homo sapiens
MLNPFIYSI

SEQ ID NO: 167 - protein, 9 aa, Homo sapiens
FLQKDIFEI

SEQ ID NO: 168 - protein, 9 aa, Homo sapiens
FLKKEIYEI

SEQ ID NO: 169 - protein, 9 aa, Homo sapiens
TMNKHLYTI

SEQ ID NO: 170 - protein, 9 aa, Homo sapiens
RLIKFIYNI

SEQ ID NO: 171 - protein, 9 aa, Homo sapiens
FLKKYLYEI

SEQ ID NO: 172 - protein, 9 aa, Homo sapiens
FMNKFIYEI

SEQ ID NO: 173 - protein, 9 aa, Homo sapiens
RMNGFIDQI

SEQ ID NO: 174 - protein, 9 aa, Homo sapiens
SMQQFLYEI

SEQ ID NO: 175 - protein, 9 aa, Homo sapiens
FQVKKIYEL

SEQ ID NO: 176 - protein, 9 aa, Homo sapiens
TLNKFIEEL

SEQ ID NO: 177 - protein, 9 aa, Homo sapiens
KLNKIISEI

SEQ ID NO: 178 - protein, 9 aa, Homo sapiens
RMNGIIYEI

SEQ ID NO: 179 - protein, 9 aa, Homo sapiens
ILNKFIPDI

SEQ ID NO: 180 - protein, 9 aa, Homo sapiens
FMAVFILEV

SEQ ID NO: 181 - protein, 9 aa, Homo sapiens
KINQFIEEI

SEQ ID NO: 182 - protein, 9 aa, Homo sapiens
ILNKFIPDI

SEQ ID NO: 183 - protein, 9 aa, Homo sapiens
SLLMWITQV

SEQ ID NO: 184 - protein, 9 aa, Homo sapiens
SLLMISENV

SEQ ID NO: 185 - protein, 9 aa, Homo sapiens
SLLLWISGA

SEQ ID NO: 186 - protein, 9 aa, Homo sapiens
SLLKDISQK

SEQ ID NO: 187 - protein, 9 aa, Homo sapiens
SLCVLITAV

SEQ ID NO: 188 - protein, 9 aa, Homo sapiens
SLLHAGTQS

SEQ ID NO: 189 - protein, 9 aa, Homo sapiens
SLRHIIAQV

SEQ ID NO: 190 - protein, 9 aa, Homo sapiens
SFLNWLTMV

SEQ ID NO: 191 - protein, 9 aa, Homo sapiens
SALWRWTQV

SEQ ID NO: 192 - protein, 9 aa, Homo sapiens
SLQMSITWQ

SEQ ID NO: 193 - protein, 9 aa, Homo sapiens
FLLMFIKQL

SEQ ID NO: 194 - protein, 9 aa, Homo sapiens
SSLSRIPQV

SEQ ID NO: 195 - protein, 9 aa, Homo sapiens
SLLYWTDVV

SEQ ID NO: 196 - protein, 9 aa, Homo sapiens
SNLSSDTQV

SEQ ID NO: 197 - protein, 9 aa, Homo sapiens
EQLMSITQE

SEQ ID NO: 198 - protein, 9 aa, Homo sapiens
SLCMVITIY

SEQ ID NO: 199 - protein, 9 aa, Homo sapiens
GLRMWIKQV

SEQ ID NO: 200 - protein, 9 aa, Homo sapiens
SLLMKMRSV

SEQ ID NO: 201 - protein, 9 aa, Homo sapiens
SLLEPETQD

SEQ ID NO: 202 - protein, 9 aa, Homo sapiens
SLGMNITSS

SEQ ID NO: 203 - protein, 9 aa, Homo sapiens
SLSMGITMM

SEQ ID NO: 204 - protein, 9 aa, Homo sapiens
LLLCDGTQV

SEQ ID NO: 205 - protein, 9 aa, Homo sapiens
SVPMQGTQV

SEQ ID NO: 206 - protein, 9 aa, Homo sapiens
SLKLTSTQV

SEQ ID NO: 207 - protein, 9 aa, Homo sapiens
SLHLTETQV

SEQ ID NO: 208 - protein, 9 aa, Homo sapiens
SLYMVVPLV

SEQ ID NO: 209 - protein, 9 aa, Homo sapiens
SLLMERLSV

SEQ ID NO: 210 - protein, 9 aa, Homo sapiens
SLLLQSTQN

SEQ ID NO: 211 - protein, 9 aa, Homo sapiens
SLLDIIEKV

SEQ ID NO: 212 - protein, 9 aa, Homo sapiens
SLLIAIKPV

SEQ ID NO: 213 - protein, 9 aa, Homo sapiens
DLLEWIEQT

SEQ ID NO: 214 - protein, 9 aa, Homo sapiens
QLLMSCPQV

SEQ ID NO: 215 - protein, 9 aa, Homo sapiens
SSLEDITYV

SEQ ID NO: 216 - protein, 9 aa, Homo sapiens
SLRKMIRQE

SEQ ID NO: 217 - protein, 9 aa, Homo sapiens
SLLMEWLSV

SEQ ID NO: 218 - protein, 9 aa, Homo sapiens
PLLMCKTQA

SEQ ID NO: 219 - protein, 9 aa, Homo sapiens
SLESWITAG

SEQ ID NO: 220 - protein, 9 aa, Homo sapiens
TLLMCIVTV

SEQ ID NO: 221 - protein, 9 aa, Homo sapiens
SLPECITQF

SEQ ID NO: 222 - protein, 9 aa, Homo sapiens
SLLIVPTSV

SEQ ID NO: 223 - protein, 9 aa, Homo sapiens
SLDCWITDK

SEQ ID NO: 224 - protein, 9 aa, Homo sapiens
SLLQDITMI

SEQ ID NO: 225 - protein, 9 aa, Homo sapiens
QLSTVITQV

SEQ ID NO: 226 - protein, 9 aa, Homo sapiens
NLLPSITDV

SEQ ID NO: 227 - protein, 9 aa, Homo sapiens
SLLIVPTSV

SEQ ID NO: 228 - protein, 9 aa, Homo sapiens
SLLIVPTSV

SEQ ID NO: 229 - protein, 9 aa, Homo sapiens
SLLLLVTSV

SEQ ID NO: 230 - protein, 9 aa, Homo sapiens
SLDALITHV

SEQ ID NO: 231 - protein, 9 aa, Homo sapiens
SLDALITHV

SEQ ID NO: 232 - protein, 9 aa, Homo sapiens
WLLNDIFQV

SEQ ID NO: 233 - protein, 9 aa, Homo sapiens
FLLMFIKQL

SEQ ID NO: 234 - protein, 9 aa, Homo sapiens
SLLQSILQL

SEQ ID NO: 235 - protein, 9 aa, Homo sapiens
SLPFLIYQV

SEQ ID NO: 236 - protein, 9 aa, Homo sapiens
SGLLNITKV

SEQ ID NO: 237 - protein, 9 aa, Homo sapiens
SLLGWILSI

SEQ ID NO: 238 - protein, 9 aa, Homo sapiens
SLLKHMLQV

SEQ ID NO: 239 - protein, 9 aa, Homo sapiens
SLRHIIAQV

SEQ ID NO: 240 - protein, 9 aa, Homo sapiens
SLLDSSNQV

SEQ ID NO: 241 - protein, 9 aa, Homo sapiens
SLFKYITVV

SEQ ID NO: 242 - protein, 9 aa, Homo sapiens
SVLGAITSV

SEQ ID NO: 243 - protein, 9 aa, Homo sapiens
SLLELVEQV

SEQ ID NO: 244 - protein, 9 aa, Homo sapiens
KVAELVHFL

SEQ ID NO: 245 - protein, 9 aa, Homo sapiens
KMAELVHFL

SEQ ID NO: 246 - protein, 9 aa, Homo sapiens
EVDPIGHLY

SEQ ID NO: 247 - protein, 9 aa, Homo sapiens
ESDPIVAQY

SEQ ID NO: 248 - protein, 9 aa, Homo sapiens
FMNKFIYEI

SEQ ID NO: 249 - protein, 9 aa, Homo sapiens
ILNKFIPDI

SEQ ID NO: 250 - protein, 9 aa, Homo sapiens
SLLMWITQV